European Patent Specification EP 3 315 510 B1, published February 19, 2025. Title: Modified Chemokine Peptide. Applicant: RISE TECHNOLOGY CO LTD. The sequence listing filed with the application follows.

SEQUENCE LISTING (12 sequences)

SEQ ID NO: 1 - protein, 72 aa, Artificial Sequence
  Modified ELR-CXC Chemokine
GSKELRCQCIRTYSKPFHPKFIKELRVIESPPHCANTEIIVKLSDGRELCLDPKENWVQRVVEKFLKRAENS

SEQ ID NO: 2 - protein, 72 aa, Homo sapiens
SAKELRCQCIKTYSKPFHPKFIKELRVIESGPHCANTEIIVKLSDGRELCLDPKENWVQRVVEKFLKRAENS

SEQ ID NO: 3 - protein, 74 aa, Homo sapiens
GASVATELRCQCLQTLQGIHPKNIQSVNVKSPGPHCAQTEVIATLKNGRKACLNPASPIVKKIIEKMLNSDKSN

SEQ ID NO: 4 - protein, 74 aa, Homo sapiens
GAPLATELRCQCLQTLQGIHLKNIQSVKVKSPGPHCAQTEVIATLKNGQKACLNPASPMVKKIIEKMLKNGKSN

SEQ ID NO: 5 - protein, 74 aa, Homo sapiens
GASVVTELRCQCLQTLQGIHLKNIQSVNVRSPGPHCAQTEVIATLKNGKKACLNPASPMVQKIIEKILNKGSTN

SEQ ID NO: 6 - protein, 73 aa, Homo sapiens
AVLRELRCVCLQTTQGVHPKMISNLQVFAIGPQCSKVEVVASLKNGKEICLDPEAPFLKKVIQKILDGGNKEN

SEQ ID NO: 7 - protein, 74 aa, Homo sapiens
SAVLTELRCTCLRVTLRVNPKTIGKLQVFPAGPQCSKVEVVASLKNGKQVCLDPEAPFLKKVIQKILDSGNKKN

SEQ ID NO: 8 - protein, 74 aa, Homo sapiens
SDLYAELRCMCIKTTSGIHPKNIQSLEVIGKGTHCNQVEVIATLKDGRKICLDPDAPRIKKIVQKKLAGDESAD

SEQ ID NO: 9 - protein, 73 aa, Artificial Sequence
  Modified ELR-CXC Chemokine
SAKELRCQACIRTYSKPFHPKFIKELRVIESGPHCANTEIIVKLSDGRELCLDPKENWVQRVVEKFLKRAENS

SEQ ID NO: 10 - protein, 72 aa, Artificial Sequence
  Modified ELR-CXC Chemokine
SAKELRCQCIKTYSKPLHPKFIKELRVIPASQFCANTEIIVKLSDGRELCLDPKENWVQRVVEKFLKRAENS

SEQ ID NO: 11 - protein, 71 aa, Artificial Sequence
  Modified ELR-CXC Chemokine
SAKELRCCIRTYSKPLHPKFIKELRVIPASQFCANTEIIVKLSDGRELCLDPKENWVQRVVEKFLKAAENS

SEQ ID NO: 12 - protein, 72 aa, Artificial Sequence
  Modified ELR-CXC Chemokine
GSKELRCQCIRTYSKPLHPKFIKELRVIPASQFCANTEIIVKLSDGRELCLDPKENWVQRVVEKFLKRAENS